European Patent Application EP 4 328 317 A1, published February 28, 2024. Title: Microorganisms producing carotenoids. Applicant: ENEOS Corporation. The sequence listing filed with the application follows.

SEQUENCE LISTING (7 sequences)

SEQ ID NO: 1 - DNA, 729 bp, Paracoccus carotinifaciens
atgagcgcacatgccctgcccaaggcagatctgaccgccaccagtttgatcgtctcgggcggcatcatcgccgcgtggctggccctgcatgtgcatgcgctgtggtttctggacgcggcggcgcatcccatcctggcggtcgcgaatttcctggggctgacctggctgtcggtcggtctgttcatcatcgcgcatgacgcgatgcatgggtcggtcgtgccggggcgcccgcgcgccaatgcggcgatgggccagcttgtcctgtggctgtatgccggattttcctggcgcaagatgatcgtcaagcacatggcccatcatcgccatgccggaaccgacgacgacccagatttcgaccatggcggcccggtccgctggtacgcccgcttcatcggcacctatttcggctggcgcgaggggctgctgctgcccgtcatcgtgacggtctatgcgctgatgttgggggatcgctggatgtacgtggtcttctggccgttgccgtcgatcctggcgtcgatccagctgttcgtgttcggcacttggctgccgcaccgccccggccacgacgcgttcccggaccgccacaatgcgcggtcgtcgcggatcagcgaccccgtgtcgctgctgacctgctttcactttggcggttatcatcacgaacaccacctgcacccgacggtgccttggtggcgcctgcccagcacccgcaccaagggggacaccgcatga

SEQ ID NO: 2 - protein, 242 aa, Paracoccus carotinifaciens
MSAHALPKADLTATSLIVSGGIIAAWLALHVHALWFLDAAAHPILAVANFLGLTWLSVGLFIIAHDAMHGSVVPGRPRANAAMGQLVLWLYAGFSWRKMIVKHMAHHRHAGTDDDPDFDHGGPVRWYARFIGTYFGWREGLLLPVIVTVYALMLGDRWMYVVFWPLPSILASIQLFVFGTWLPHRPGHDAFPDRHNARSSRISDPVSLLTCFHFGGYHHEHHLHPTVPWWRLPSTRTKGDTA

SEQ ID NO: 3 - DNA, 729 bp, Paracoccus carotinifaciens
atgagcgcacatgccctgcccaaggcagatctgaccgccaccagtttgatcgtctcgggcggcatcatcgccgcgtggctggccctgcatgtgcatgcgctgtggtttctggacgcggcggcgcatcccatcctggcggtcgcgaatttcctggggctgacctggctgtcggtcggtctgttcatcatcgcgcatgacgcgatgcatgggtcggtcgtgccggggcgcccgcgcgccaatgcggcgatgggccagcttgtcctgtggctgtatgccggattttcctggcgcaagatgatcgtcaagcacatggcccatcatcgccatgccggaaccgacgacgacccagatttcgaccatggcggcccggtccgctggtacgcccgcttcatcggcacctatttcggctggcgcgaggggctgctgctgcccgtcatcgtgacggtctatgcgctgatgttgggggatcgctggatgtacgtggtcttctggccgttgccgtcgatcctggcgtcgatccagctgttcgtgttcggcacttggctgccgcaccgccccggccacgacgcgttcccggaccgccacaatgcgcggtcgtcgcggatcagcgaccccgtgtcgctgctgacctgctttcactttggcggttatcatcacgaacaccacctgcacccgacggtgccttggtgacgcctgcccagcacccgcaccaagggggacaccgcatga

SEQ ID NO: 4 - protein, 229 aa, Paracoccus carotinifaciens
MSAHALPKADLTATSLIVSGGIIAAWLALHVHALWFLDAAAHPILAVANFLGLTWLSVGLFIIAHDAMHGSVVPGRPRANAAMGQLVLWLYAGFSWRKMIVKHMAHHRHAGTDDDPDFDHGGPVRWYARFIGTYFGWREGLLLPVIVTVYALMLGDRWMYVVFWPLPSILASIQLFVFGTWLPHRPGHDAFPDRHNARSSRISDPVSLLTCFHFGGYHHEHHLHPTVPW

SEQ ID NO: 5 - DNA, 729 bp, Paracoccus carotinifaciens
atgagcgcacatgccctgcccaaggcagatctgaccgccaccagtttgatcgtctcgggcggcatcatcgccgcgtggctggccctgcatgtgcatgcgctgtggtttctggacgcggcggcgcatcccatcctggcggtcgcgaatttcctggggctgacctggctgtcggtcggtctgttcatcatcgcgtatgacgcgatgcatgggtcggtcgtgccggggcgcccgcgcgccaatgcggcgatgggccagcttgtcctgtggctgtatgccggattttcctggcgcaagatgatcgtcaagcacatggcccatcatcgccatgccggaaccgacgacgacccagatttcgaccatggcggcccggtccgctggtacgcccgcttcatcggcacctatttcggctggcgcgaggggctgctgctgcccgtcatcgtgacggtctatgcgctgatgttgggggatcgctggatgtacgtggtcttctggccgttgccgtcgatcctggcgtcgatccagctgttcgtgttcggcacttggctgccgcaccgccccggccacgacgcgttcccggaccgccacaatgcgcggtcgtcgcggatcagcgaccccgtgtcgctgctgacctgctttcactttggcggttatcatcacgaacaccacctgcacccgacggtgccttggtggcgcctgcccagcacccgcaccaagggggacaccgcatga

SEQ ID NO: 6 - protein, 242 aa, Paracoccus carotinifaciens
MSAHALPKADLTATSLIVSGGIIAAWLALHVHALWFLDAAAHPILAVANFLGLTWLSVGLFIIAYDAMHGSVVPGRPRANAAMGQLVLWLYAGFSWRKMIVKHMAHHRHAGTDDDPDFDHGGPVRWYARFIGTYFGWREGLLLPVIVTVYALMLGDRWMYVVFWPLPSILASIQLFVFGTWLPHRPGHDAFPDRHNARSSRISDPVSLLTCFHFGGYHHEHHLHPTVPWWRLPSTRTKGDTA

SEQ ID NO: 7 - DNA, 1452 bp, Paracoccus carotinifaciens
  misc_feature (1350)..(1350): n is a, c, g, or t
agtttgatcctggctcagaacgaacgctggcggcaggcttaacacatgcaagtcgagcgagaccttcgggtctagcggcggacgggtgagtaacgcgtgggaacgtgcccttctctacggaatagccccgggaaactgggagtaataccgtatacgccctttgggggaaagatttatcggagaaggatcggcccgcgttggattaggtagttggtggggtaatggcccaccaagccgacgatccatagctggtttgagaggatgatcagccacactgggactgagacacggcccagactcctacgggaggcagcagtggggaatcttagacaatgggggcaaccctgatctagccatgccgcgtgagtgatgaaggccttagggttgtaaagctctttcagctgggaagataatgacggtaccagcagaagaagccccggctaactccgtgccagcagccgcggtaatacggagggggctagcgttgttcggaattactgggcgtaaagcgcacgtaggcggactggaaagtcagaggtgaaatcccagggctcaaccttggaactgcctttgaaactatcagtctggagttcgagagaggtgagtggaattccgagtgtagaggtgaaattcgtagatattcggaggaacaccagtggcgaaggcggctcactggctcgatactgacgctgaggtgcgaaagcgtggggagcaaacaggattagataccctggtagtccacgccgtaaacgatgaatgccagacgtcggcaagcatgcttgtcggtgtcacacctaacggattaagcattccgcctggggagtacggtcgcaagattaaaactcaaaggaattgacgggggcccgcacaagcggtggagcatgtggtttaattcgaagcaacgcgcagaaccttaccaacccttgacatggcaggaccgctggagagattcagctttctcgtaagagacctgcacacaggtgctgcatggctgtcgtcagctcgtgtcgtgagatgttcggttaagtccggcaacgagcgcaacccacgtccctagttgccagcaattcagttgggaactctatggaaactgccgatgataagtcggaggaaggtgtggatgacgtcaagtcctcatgggccttacgggttgggctacacacgtgctacaatggtggtgacagtgggttaatccccaaaagccatctcagttcggattgtcctctgcaactcgagggcatgaagttggaatcgctagtaatcgcggaacagcatgccgcggtgaatacgttcccgggccttgtacacaccgcccgtcacaccatgggagttggttctacccgacgacgntgcgctaaccttcggggggcaggcggccacggtaggatcagcgactggggtgaagtcgtaacaaggtagccgtaggggaacctgcggctggatcacctcctt